European Patent Application EP 4 400 114 A1, published July 17, 2024. Title: Improvement of tumor immunogenicity by a splicing modulator. Applicant: Kyoto University. The sequence listing filed with the application follows.

SEQUENCE LISTING (36 sequences)

SEQ ID NO: 1 - protein, 9 aa, Mus musculus
MALSNKAYV

SEQ ID NO: 2 - protein, 9 aa, Mus musculus
RNRSHIFPL

SEQ ID NO: 3 - protein, 8 aa, Mus musculus
SILGFTMV

SEQ ID NO: 4 - protein, 9 aa, Mus musculus
SLLLLYLQL

SEQ ID NO: 5 - protein, 9 aa, Mus musculus
KQQELFVLL

SEQ ID NO: 6 - protein, 10 aa, Mus musculus
SQPLPNKIGF

SEQ ID NO: 7 - protein, 11 aa, Mus musculus
TSLQNYKCTEC

SEQ ID NO: 8 - protein, 9 aa, Mus musculus
KSLDNKGHL

SEQ ID NO: 9 - protein, 11 aa, Mus musculus
SLSSNTSYGEI

SEQ ID NO: 10 - protein, 8 aa, Mus musculus
QSFSQERL

SEQ ID NO: 11 - protein, 8 aa, Mus musculus
RVNFFAIL

SEQ ID NO: 12 - protein, 9 aa, Mus musculus
QTQSNTEEI

SEQ ID NO: 13 - protein, 8 aa, Mus musculus
IIYQKAKV

SEQ ID NO: 14 - protein, 9 aa, Mus musculus
STLHLSQAL

SEQ ID NO: 15 - protein, 8 aa, Mus musculus
DGPLFLKL

SEQ ID NO: 16 - protein, 8 aa, Mus musculus
TAPSFLPL

SEQ ID NO: 17 - protein, 9 aa, Mus musculus
AAGKKTQEL

SEQ ID NO: 18 - protein, 8 aa, Mus musculus
SLYKICKM

SEQ ID NO: 19 - protein, 9 aa, Mus musculus
TELLSHTPL

SEQ ID NO: 20 - protein, 9 aa, Mus musculus
FAKQEIELL

SEQ ID NO: 21 - protein, 9 aa, Mus musculus
VQFSAIDKL

SEQ ID NO: 22 - protein, 8 aa, Mus musculus
SSALFSYV

SEQ ID NO: 23 - DNA, 22 bp, synthetic construct
  source 1..22: mol_type = other DNA
ttcctgtgagaaagaggtggag

SEQ ID NO: 24 - DNA, 25 bp, synthetic construct
  source 1..25: mol_type = other DNA
cacaaacataagccttattgctcag

SEQ ID NO: 25 - DNA, 25 bp, synthetic construct
  source 1..25: mol_type = other DNA
cactttagtgaagagaccaagcaag

SEQ ID NO: 26 - DNA, 24 bp, synthetic construct
  source 1..24: mol_type = other DNA
tcatacatgcttgttgtggcagag

SEQ ID NO: 27 - DNA, 22 bp, synthetic construct
  source 1..22: mol_type = other DNA
catgggtaccgagaaggaagag

SEQ ID NO: 28 - DNA, 19 bp, synthetic construct
  source 1..19: mol_type = other DNA
tccaatggggtcccagaac

SEQ ID NO: 29 - DNA, 20 bp, synthetic construct
  source 1..20: mol_type = other DNA
aaactggagatggggactta

SEQ ID NO: 30 - DNA, 20 bp, synthetic construct
  source 1..20: mol_type = other DNA
tgaggattctcctggcaatg

SEQ ID NO: 31 - DNA, 22 bp, synthetic construct
  source 1..22: mol_type = other DNA
ccaagtgagaaagttcctggag

SEQ ID NO: 32 - DNA, 21 bp, synthetic construct
  source 1..21: mol_type = other DNA
gaggacaaagagctcctgctg

SEQ ID NO: 33 - DNA, 22 bp, synthetic construct
  source 1..22: mol_type = other DNA
ccagagaatgaggaagtggaag

SEQ ID NO: 34 - DNA, 20 bp, synthetic construct
  source 1..20: mol_type = other DNA
gtaaatccaatcttgtttgg

SEQ ID NO: 35 - DNA, 20 bp, synthetic construct
  source 1..20: mol_type = other DNA
tctttgcagctccttcgttg

SEQ ID NO: 36 - DNA, 19 bp, synthetic construct
  source 1..19: mol_type = other DNA
ggcctcgtcacccacatag